European Patent Application EP 4 245 767 A1, published September 20, 2023. Title: MODIFIED ENVELOPE PROTEIN OF HUMAN IMMUNODEFICIENCY VIRUS AND USE THEREOF. Applicant: XIAMEN UNIVERSITY XIAMEN INNOVAX BIOTECH CO., LTD. The sequence listing filed with the application follows.

SEQUENCE LISTING (41 sequences)

SEQ ID NO: 1 - protein, 659 aa, Artificial Sequence
  BG505 TST
MDAMKRGLCCVLLLCGAVFVSPSQEIHARFRRGARAENLAVGIGAVFLGFLGAAGSTMGAASMTLTVQARNLLSGIVQQQSNLLRAIEAQQHLLKLTVWGIKQLQARVLAVERYLRDQQLLGIWGCSGKLICTTNVPNLWVTVYYGVPVWKDAETTLFCASDAKAYETEKHNVWATHACVPTDPNPQEIHLENVTEEFNMWKNNMVEQMHTDIISLWDQSLKPCVKLTPLCVTLQCTNVTNNITDDMRGELKNCSFNMTTELRDKKQKVYSLFYRLDVVQINENQGNRSNNSNKEYRLINCNTSAITQACPKVSFEPIPIHYCAPAGFAILKCKDKKFNGTGPCPSVSTVQCTHGIKPVVSTQLLLNGSLAEEEVMIRSENITNNAKNILVQFNTPVQINCTRPNNNTRKSIRIGPGQAFYATGDIIGDIRQAHCNVSKATWNETLGKVVKQLRKHFGNNTIIRFANSSGGDLEVTTHSFNCGGEFFYCNTSGLFNSTWISNTSVQGSNSTGSNDSITLPCRIKQIINMWQRIGQAMYAPPIQGVIRCVSNITGLILTRDGGSTNSTTETFRPGGGDMRDNWRSELYKYKVVKIEPLGVAPTRRNLSEIWDNMTWLQWDKEISNYTQIIYGLLEESQNQQEKNEQDLLALDHHHHHHHH

SEQ ID NO: 2 - protein, 660 aa, Artificial Sequence
  NL4-3 TST
MDAMKRGLCCVLLLCGAVFVSPSQEIHARFRRGARAENLAVGIGALFLGFLGAAGSTMGAASMTLTVQARQLLSDIVQQQNNLLRAIEAQQHLLQLTVWGIKQLQARILAVERYLKDQQLLGIWGCSGKLICTTAVPNLWVTVYYGVPVWKEATTTLFCASDAKAYDTEVHNVWATHACVPTDPNPQEVVLVNVTENFNMWKNDMVEQMHEDIISLWDQSLKPCVKLTPLCVSLKCTDLKNDTNTNSSSGRMIMEKGEIKNCSFNISTSIRDKVQKEYAFFYKLDIVPIDNTSYRLISCNTSVITQACPKVSFEPIPIHYCAPAGFAILKCNNKTFNGTGPCTNVSTVQCTHGIRPVVSTQLLLNGSLAEEDVVIRSANFTDNAKTIIVQLNTSVEINCTRPNNNTRKSIRIQRGPGRAFVTIGKIGNMRQAHCNISRAKWNATLKQIASKLREQFGNNKTIIFKQSSGGDPEIVTHSFNCGGEFFYCNSTQLFNSTWFNSTWSTEGSNNTEGSDTITLPCRIKQFINMWQEVGKAMYAPPISGQIRCSSNITGLLLTRDGGNNNNGSEIFRPGGGDMRDNWRSELYKYKVVKIEPLGVAPTKKSLEQIWNNMTWMEWDREINNYTSLIHSLIEESQNQQEKNEQELLELDKHHHHHHHH

SEQ ID NO: 3 - protein, 659 aa, Artificial Sequence
  BG505 TSTIP
MDAMKRGLCCVLLLCGAVFVSPSQEIHARFRRGARAENLAVGIGAVFLGFLGAAGSTMGAASMTLTVQARNLLSGIVQQQSNLLRAPEAQQHLLKLTVWGIKQLQARVLAVERYLRDQQLLGIWGCSGKLICTTNVPNLWVTVYYGVPVWKDAETTLFCASDAKAYETEKHNVWATHACVPTDPNPQEIHLENVTEEFNMWKNNMVEQMHTDIISLWDQSLKPCVKLTPLCVTLQCTNVTNNITDDMRGELKNCSFNMTTELRDKKQKVYSLFYRLDVVQINENQGNRSNNSNKEYRLINCNTSAITQACPKVSFEPIPIHYCAPAGFAILKCKDKKFNGTGPCPSVSTVQCTHGIKPVVSTQLLLNGSLAEEEVMIRSENITNNAKNILVQFNTPVQINCTRPNNNTRKSIRIGPGQAFYATGDIIGDIRQAHCNVSKATWNETLGKVVKQLRKHFGNNTIIRFANSSGGDLEVTTHSFNCGGEFFYCNTSGLFNSTWISNTSVQGSNSTGSNDSITLPCRIKQIINMWQRIGQAMYAPPIQGVIRCVSNITGLILTRDGGSTNSTTETFRPGGGDMRDNWRSELYKYKVVKIEPLGVAPTRRNLSEIWDNMTWLQWDKEISNYTQIIYGLLEESQNQQEKNEQDLLALDHHHHHHHH

SEQ ID NO: 4 - protein, 660 aa, Artificial Sequence
  NL4-3 TSTIP
MDAMKRGLCCVLLLCGAVFVSPSQEIHARFRRGARAENLAVGIGALFLGFLGAAGSTMGAASMTLTVQARQLLSDIVQQQNNLLRAPEAQQHLLQLTVWGIKQLQARILAVERYLKDQQLLGIWGCSGKLICTTAVPNLWVTVYYGVPVWKEATTTLFCASDAKAYDTEVHNVWATHACVPTDPNPQEVVLVNVTENFNMWKNDMVEQMHEDIISLWDQSLKPCVKLTPLCVSLKCTDLKNDTNTNSSSGRMIMEKGEIKNCSFNISTSIRDKVQKEYAFFYKLDIVPIDNTSYRLISCNTSVITQACPKVSFEPIPIHYCAPAGFAILKCNNKTFNGTGPCTNVSTVQCTHGIRPVVSTQLLLNGSLAEEDVVIRSANFTDNAKTIIVQLNTSVEINCTRPNNNTRKSIRIQRGPGRAFVTIGKIGNMRQAHCNISRAKWNATLKQIASKLREQFGNNKTIIFKQSSGGDPEIVTHSFNCGGEFFYCNSTQLFNSTWFNSTWSTEGSNNTEGSDTITLPCRIKQFINMWQEVGKAMYAPPISGQIRCSSNITGLLLTRDGGNNNNGSEIFRPGGGDMRDNWRSELYKYKVVKIEPLGVAPTKKSLEQIWNNMTWMEWDREINNYTSLIHSLIEESQNQQEKNEQELLELDKHHHHHHHH

SEQ ID NO: 5 - protein, 673 aa, Artificial Sequence
  BG505 TSTIP full
MDAMKRGLCCVLLLCGAVFVSPSQEIHARFRRGARAENLAVGIGAVFLGFLGAAGSTMGAASMTLTVQARNLLSGIVQQQSNLLRAPEAQQHLLKLTVWGIKQLQARVLAVERYLRDQQLLGIWGCSGKLICTTNVPWNSSWSNNLWVTVYYGVPVWKDAETTLFCASDAKAYETEKHNVWATHACVPTDPNPQEIHLENVTEEFNMWKNNMVEQMHTDIISLWDQSLKPCVKLTPLCVTLQCTNVTNNITDDMRGELKNCSFNMTTELRDKKQKVYSLFYRLDVVQINENQGNRSNNSNKEYRLINCNTSAITQACPKVSFEPIPIHYCAPAGFAILKCKDKKFNGTGPCPSVSTVQCTHGIKPVVSTQLLLNGSLAEEEVMIRSENITNNAKNILVQFNTPVQINCTRPNNNTRKSIRIGPGQAFYATGDIIGDIRQAHCNVSKATWNETLGKVVKQLRKHFGNNTIIRFANSSGGDLEVTTHSFNCGGEFFYCNTSGLFNSTWISNTSVQGSNSTGSNDSITLPCRIKQIINMWQRIGQAMYAPPIQGVIRCVSNITGLILTRDGGSTNSTTETFRPGGGDMRDNWRSELYKYKVVKIEPLGVAPTRAKRRVVGRNLSEIWDNMTWLQWDKEISNYTQIIYGLLEESQNQQEKNEQDLLALDHHHHHHHH

SEQ ID NO: 6 - protein, 686 aa, Artificial Sequence
  NL4-3 TSTIP full
MDAMKRGLCCVLLLCGAVFVSPSQEIHARFRRGARAENLREKRAVGIGALFLGFLGAAGSTMGAASMTLTVQARQLLSDIVQQQNNLLRAPEAQQHLLQLTVWGIKQLQARILAVERYLKDQQLLGIWGCSGKLICTTAVPWNASWSNNLWVTVYYGVPVWKEATTTLFCASDAKAYDTEVHNVWATHACVPTDPNPQEVVLVNVTENFNMWKNDMVEQMHEDIISLWDQSLKPCVKLTPLCVSLKCTDLKNDTNTNSSSGRMIMEKGEIKNCSFNISTSIRDKVQKEYAFFYKLDIVPIDNTSYRLISCNTSVITQACPKVSFEPIPIHYCAPAGFAILKCNNKTFNGTGPCTNVSTVQCTHGIRPVVSTQLLLNGSLAEEDVVIRSANFTDNAKTIIVQLNTSVEINCTRPNNNTRKSIRIQRGPGRAFVTIGKIGNMRQAHCNISRAKWNATLKQIASKLREQFGNNKTIIFKQSSGGDPEIVTHSFNCGGEFFYCNSTQLFNSTWFNSTWSTEGSNNTEGSDTITLPCRIKQFINMWQEVGKAMYAPPISGQIRCSSNITGLLLTRDGGNNNNGSEIFRPGGGDMRDNWRSELYKYKVVKIEPLGVAPTKAKRRVVQKSLEQIWNNMTWMEWDREINNYTSLIHSLIEESQNQQEKNEQELLELDKGSGSGGSGHHHHHHHH

SEQ ID NO: 7 - protein, 669 aa, Artificial Sequence
  BG505 TSTIP G1
MDAMKRGLCCVLLLCGAVFVSPSQEIHARFRRGARAENLAVGIGAVFLGFLGAAGSTMGAASMTLTVQARNLLSGIVQQQSNLLRAPEAQQHLLKLTVWGIKQLQARVLAVERYLRDQQLLGIWGCSGKLICTTNVPGGGGSNLWVTVYYGVPVWKDAETTLFCASDAKAYETEKHNVWATHACVPTDPNPQEIHLENVTEEFNMWKNNMVEQMHTDIISLWDQSLKPCVKLTPLCVTLQCTNVTNNITDDMRGELKNCSFNMTTELRDKKQKVYSLFYRLDVVQINENQGNRSNNSNKEYRLINCNTSAITQACPKVSFEPIPIHYCAPAGFAILKCKDKKFNGTGPCPSVSTVQCTHGIKPVVSTQLLLNGSLAEEEVMIRSENITNNAKNILVQFNTPVQINCTRPNNNTRKSIRIGPGQAFYATGDIIGDIRQAHCNVSKATWNETLGKVVKQLRKHFGNNTIIRFANSSGGDLEVTTHSFNCGGEFFYCNTSGLFNSTWISNTSVQGSNSTGSNDSITLPCRIKQIINMWQRIGQAMYAPPIQGVIRCVSNITGLILTRDGGSTNSTTETFRPGGGDMRDNWRSELYKYKVVKIEPLGVAPTRGGGGSRNLSEIWDNMTWLQWDKEISNYTQIIYGLLEESQNQQEKNEQDLLALDHHHHHHHH

SEQ ID NO: 8 - protein, 682 aa, Artificial Sequence
  NL4-3 TSTIP G1
MDAMKRGLCCVLLLCGAVFVSPSQEIHARFRRGARAENLREKRAVGIGALFLGFLGAAGSTMGAASMTLTVQARQLLSDIVQQQNNLLRAPEAQQHLLQLTVWGIKQLQARILAVERYLKDQQLLGIWGCSGKLICTTAVPGGGGSNLWVTVYYGVPVWKEATTTLFCASDAKAYDTEVHNVWATHACVPTDPNPQEVVLVNVTENFNMWKNDMVEQMHEDIISLWDQSLKPCVKLTPLCVSLKCTDLKNDTNTNSSSGRMIMEKGEIKNCSFNISTSIRDKVQKEYAFFYKLDIVPIDNTSYRLISCNTSVITQACPKVSFEPIPIHYCAPAGFAILKCNNKTFNGTGPCTNVSTVQCTHGIRPVVSTQLLLNGSLAEEDVVIRSANFTDNAKTIIVQLNTSVEINCTRPNNNTRKSIRIQRGPGRAFVTIGKIGNMRQAHCNISRAKWNATLKQIASKLREQFGNNKTIIFKQSSGGDPEIVTHSFNCGGEFFYCNSTQLFNSTWFNSTWSTEGSNNTEGSDTITLPCRIKQFINMWQEVGKAMYAPPISGQIRCSSNITGLLLTRDGGNNNNGSEIFRPGGGDMRDNWRSELYKYKVVKIEPLGVAPTKGGGGSKSLEQIWNNMTWMEWDREINNYTSLIHSLIEESQNQQEKNEQELLELDKGSGSGGSGHHHHHHHH

SEQ ID NO: 9 - protein, 679 aa, Artificial Sequence
  BG505 TSTIP G2
MDAMKRGLCCVLLLCGAVFVSPSQEIHARFRRGARAENLAVGIGAVFLGFLGAAGSTMGAASMTLTVQARNLLSGIVQQQSNLLRAPEAQQHLLKLTVWGIKQLQARVLAVERYLRDQQLLGIWGCSGKLICTTNVPGGGGSGGGGSNLWVTVYYGVPVWKDAETTLFCASDAKAYETEKHNVWATHACVPTDPNPQEIHLENVTEEFNMWKNNMVEQMHTDIISLWDQSLKPCVKLTPLCVTLQCTNVTNNITDDMRGELKNCSFNMTTELRDKKQKVYSLFYRLDVVQINENQGNRSNNSNKEYRLINCNTSAITQACPKVSFEPIPIHYCAPAGFAILKCKDKKFNGTGPCPSVSTVQCTHGIKPVVSTQLLLNGSLAEEEVMIRSENITNNAKNILVQFNTPVQINCTRPNNNTRKSIRIGPGQAFYATGDIIGDIRQAHCNVSKATWNETLGKVVKQLRKHFGNNTIIRFANSSGGDLEVTTHSFNCGGEFFYCNTSGLFNSTWISNTSVQGSNSTGSNDSITLPCRIKQIINMWQRIGQAMYAPPIQGVIRCVSNITGLILTRDGGSTNSTTETFRPGGGDMRDNWRSELYKYKVVKIEPLGVAPTRGGGGSGGGGSRNLSEIWDNMTWLQWDKEISNYTQIIYGLLEESQNQQEKNEQDLLALDHHHHHHHH

SEQ ID NO: 10 - protein, 692 aa, Artificial Sequence
  NL4-3 TSTIP G2
MDAMKRGLCCVLLLCGAVFVSPSQEIHARFRRGARAENLREKRAVGIGALFLGFLGAAGSTMGAASMTLTVQARQLLSDIVQQQNNLLRAPEAQQHLLQLTVWGIKQLQARILAVERYLKDQQLLGIWGCSGKLICTTAVPGGGGSGGGGSNLWVTVYYGVPVWKEATTTLFCASDAKAYDTEVHNVWATHACVPTDPNPQEVVLVNVTENFNMWKNDMVEQMHEDIISLWDQSLKPCVKLTPLCVSLKCTDLKNDTNTNSSSGRMIMEKGEIKNCSFNISTSIRDKVQKEYAFFYKLDIVPIDNTSYRLISCNTSVITQACPKVSFEPIPIHYCAPAGFAILKCNNKTFNGTGPCTNVSTVQCTHGIRPVVSTQLLLNGSLAEEDVVIRSANFTDNAKTIIVQLNTSVEINCTRPNNNTRKSIRIQRGPGRAFVTIGKIGNMRQAHCNISRAKWNATLKQIASKLREQFGNNKTIIFKQSSGGDPEIVTHSFNCGGEFFYCNSTQLFNSTWFNSTWSTEGSNNTEGSDTITLPCRIKQFINMWQEVGKAMYAPPISGQIRCSSNITGLLLTRDGGNNNNGSEIFRPGGGDMRDNWRSELYKYKVVKIEPLGVAPTKGGGGSGGGGSKSLEQIWNNMTWMEWDREINNYTSLIHSLIEESQNQQEKNEQELLELDKGSGSGGSGHHHHHHHH

SEQ ID NO: 11 - protein, 616 aa, Artificial Sequence
  25710-TSTIP
AVGIGAVFLGFLGAAGSTMGAASITLTVQARQLLSGIVQQQSNLLRAPEAQQHLLQLTVWGIKQLQTRVLAIERYLKDQQLLGIWGCSGKLICTTAVPNLWVTVYYGVPVWKEATTTLFCASDAKAYDKEVHNVWATHACVPTDPNPQEMVLGNVTENFNMWKNEMVNQMHEDVISLWDQSLKPCVKLTPLCVTLECSNVTYNESMKEVKNCSFNLTTELRDKKQKVHALFYRLDIVPLNDTEKKNSSRPYRLINCNTSAITQACPKVTFDPIPIHYCTPAGYAILKCNDKKFNGTGPCHKVSTVQCTHGIKPVVSTQLLLNGSLAEGEIIIRSENLTNNAKTIIVHLNQSVEIVCARPSNNTRTSIRIGPGQTFYATGAITGDIRQAHCNISKDKWNETLQRVGEKLAEHFPNKTIKFNSSSGGDLEITTHSFNCRGEFFYCNTSGLFNGTFNGTYVSPNSTDSNSSSIITIPCRIKQIINMWQEVGRAMYAPPIAGNITCKSNITGLLLVRDGGTGSESNKTEIFRPGGGDMRDNWRSELYKYKVVEIKPLGVAPTKRSQDDIWDNMTWMQWDKEISNYTNTIYKLLEDSQIQQEKNEKDLLALDSHHHHHHHH

SEQ ID NO: 12 - protein, 654 aa, Artificial Sequence
  X1632-TSTIP
MDAMKRGLCCVLLLCGAVFVSPSQEIHARFRRGARAIGLGTVLLGFLGTAGSTMGAASITLTVQVRQLLSGIVQQQSNLLRAPEAQQHLLQLTVWGIKQLQARVLAVERYLKDQQILGIWGCSGKLICTTNVPNLWVTVYYGVPVWEDADTTLFCASDAKAYSTESHNVWATHACVPTDPNPQEIYLENVTEDFNMWENNMVEQMQEDIISLWDESLKPCVKLTPLCVTLTCTNVTNVTDSVGTNSRLKGYKEELKNCSFNTTTEIRDKKKQEYALFYKLDIVPINDNSNNSNGYRLINCNVSTIKQACPKVSFDPIPIHYCAPAGFAILKCRDKEFNGTGTCRNVSTVQCTHGIKPVVSTQLLLNGSLAEGDIVIRSENITDNAKTIIVHLNKTVSITCTRPNNNTRKSIRIGPGQALYATGAIIGDTRQAHCNINGSEWYEMIQNVKNKLNETFKKNITFNPSSGGDLEITTHSFNCRGEFFYCNTSELFNSSHLFNGSTLSTNGTITLPCRIKQIVRMWQRVGQAMYAPPIAGNITCRSNITGLLLTRDGGTNKDTNEAETFRPGGGDMRDNWRSELYKYKVVKIKPLGVAPTRKSYSDIWDNLTWIQWEREISNYTQQIYTLLEESQNQQEKNEQELLALDKHHHHHHHH

SEQ ID NO: 13 - protein, 656 aa, Artificial Sequence
  CH119-TSTIP (BC)
MDAMKRGLCCVLLLCGAVFVSPSQEIHARFRRGARAVGIGAVFLGFLGVAGSTMGAASMTLTVQARQLLSGIVQQQSNLLRAPEAQQHLLQLTVWGIKQLQTRVLAIERYLKDQQLLGIWGCSGKLICTTAVPNLWVTVYYGVPVWKEATTTLFCASDAKAYDTEVHNVWATHACVPTDPSPQELVLENVTENFNMWKNEMVNQMHEDVISLWDQSLKPCVKLTPLCVTLECSKVSNNETDKYNGTEEMKNCSFNATTVVRDRQQKVYALFYRLDIVPLTEKNSSENSSKYYRLINCNTSAITQACPKVSFEPIPIHYCTPAGYAILKCNDKTFNGTGPCHNVSTVQCTHGIKPVVSTQLLLNGSLAEGEIIIRSENLTNNVKTILVHLNQSVEIVCTRPNNNTRKSIRIGPGQTFYATGDIIGDIRQAHCNISKWHETLKRVSEKLAEHFPNKTINFTSSSGGDLEITTHSFTCRGEFFYCNTSGLFNSTYMPNGTYLHGDTNSNSSITIPCRIKQIINMWQEVGRAMYAPPIEGNITCKSNITGLLLVRDGGTESNNTETNNTEIFRPGGGDMRDNWRSELYKYKVVEIKPLGVAPTAKSQKEIWDNMTWMQWDKEISNYTNTIYKLLEDSQNQQESNEKDLLALDHHHHHHHH

SEQ ID NO: 14 - protein, 646 aa, Artificial Sequence
  CNE8-TSTIP(AE)
MDAMKRGLCCVLLLCGAVFVSPSQEIHARFRRGARAVGIGAMIFGFLGAAGSTMGAASITLTVQARQLLSGIVQQQSNLLRAPEAQQHLLQLTVWGIKQLQARVLAVERYLKDQKFLGLWGCSGKIICTTAVPNLWVTVYYGVPVWRDADTTLFCASDAKAYDTEVHNVWATHACVPTDPNPQEIHLENVTENFNMWKNKMAEQMQEDVISLWDESLKPCVQLTPLCVTLNCTNANLNATVNASTTIGNITDEVRNCSFNTTTELRDKKQNVYALFYKLDIVPINNNSEYRLINCNTSVIKQACPKVSFDPIPIHYCAPAGYAILRCNDKNFNGTGPCKNVSSVQCTHGIKPVVSTQLLLNGSLAEDEIIIRSENLTDNVKTIIVHLNKSVEINCTRPSNNTRTSVRIGPGQVFYRTGDIIGDIRKAYCEINRTKWHETLKQVATKLREHFNKTIIFQPPSGGDIEITMHHFNCRGEFFYCNTTKLFNSTWGENTTMEGHNDTIVLPCRIKQIVNMWQGVGQAMYAPPIRGSINCVSNITGILLTRDGGTNMSNETFRPGGGNIKDNWRSELYKYKVVEIEPLGIAPTKRSYEEIWDNMTWIEWEREISNYTSQIYEILTESQNQQDRNEKDLLELDKHHHHHHHH

SEQ ID NO: 15 - protein, 647 aa, Artificial Sequence
  p246F3-TSTIP
MDAMKRGLCCVLLLCGAVFVSPSQEIHARFRRGARAVGIGAVFIGFLGAAGSTMGAASITLTVQARQLLSGIVQQQSNLLRAPEAQQHLLKLTVWGIKQLQARVLAVERYLKDQQLLGIWGCSGKLICTTNVDLWVTVYYGVPVWKDAKTTLFCASDAKAYEKEVHNVWATHACVPTDPNPQEIVMANVTEEFNMWKNNMVEQMHTDIISLWDQSLKPCVKLTPLCVTLDCKDYNYSITNNSTGMEGEIKNCSYNITTELRDKRQKVYSLFYRLDVVQINDSNDRNNSQYRLINCNTTTMTQACPKVTFDPIPIHYCAPAGFAILKCNNKTFNGKGPCNNVSSVQCTHGIKPVVSTQLLLNGSLAEKEIVIRSENLTDNVKTIIVHLNESVEINCTRPNNNTRKSVRIGPGQTFYATGDIIGNIRQAHCNVNKTEWNTALTRVSKKLKEYFPNKTIAFQPSSGGDLEITTFSFNCRGEFFYCNTSDLFNGTFNETSGQFNSTFNSTLQCRIKQIINMWQEVGQAMYAPPIAGSITCISNITGLILTRDGGNTNSTKETFRPGGGNMRDNWRSELYKYKVVKIEPLGVAPTKKSQDEIWDNMTWLQWDKEISNYTQIIYNLIEESQTQQELNERDLLALDHHHHHHHH

SEQ ID NO: 16 - protein, 836 aa, Artificial Sequence
  Bal.26-TSTIP-gp160 (AA:646-836 are transmembrane region and intracellular region)
MRVTEIRKSYQHWWRWGIMLLGMLMICNAEEKAVGIGAVLLGFLGAAGSTMGAASMTLTVQARLLLSGIVQQQNNLLRAIEAQQHLLQLTVWGIKQLQARVLAVERYLRDQQLLGPWGCSGKLICTTAVPNLWVTVYYGVPVWKEATTTLFCASDAKAYDTEVHNVWATHACVPTDPNPQEVKMENVTENFNMWKNNVVEQMHEDIISLWDQSLKPCVKLTPLCVTLNCTDLKNATNGNNTNTTSSSGGMMGGGEMKNCSFNITTNIRGKVQKEYALFYELDIVPIDNKIDSYRLISCNTSVITQACPKVSFEPIPIHYCAPAGFAILKCKDKKFNGKGPCSNVSTVQCTHGIRPVVSTQLLLNGSLAEEEVVIRSENFTNNAKIIVVQLNESVEINCTRPNNNTRKSIHIGPGRAFYTTGEIIGDIRQAHCNLSRAKWNDTLNKIVIKLREQFGNKTIVFKHSSGGDPEIVTHSFNCGGEFFYCNSTQLFNSTWNVTEESNNTVENNTITLPCRIKQIINMWQEVGRAMYAPPIRGQIRCSSNITGLLLTRDGGPEDDKTEVFRPGGGDMRDNWRSELYKYKVVKIEPLGVAPTKKSLNKIWDNMTWMEWDREINNYTSIIYSLIEESQNQQEKNEQELLELDKWASLWNWFDITKWLWYIKIFIMIVGGLIGLRIVFSVLSIVNRVRQGYSPLSFQTHLPASRGPDRPGGIEEEGGERDRDRSGPLVNGFLTLIWVDLRSLFLFSYHRLRDLLLIVTRIVELLGRRGWEVLKYWWNLLQYWSQELKNSAVSLLNTIAIAVAEGTDRVIEVVQRAVRAILHIPRRIRQGLERALL

SEQ ID NO: 17 - protein, 837 aa, Artificial Sequence
  NL4-3 TSTIP-gp160 (aa646-837 are transmembrane region and intracellular region)
MRVKEKYQHLWRWGWKWGTMLLGILMICSATEKAVGIGALFLGFLGAAGSTMGAASMTLTVQARQLLSDIVQQQNNLLRAPEAQQHLLQLTVWGIKQLQARILAVERYLKDQQLLGIWGCSGKLICTTAVPNLWVTVYYGVPVWKEATTTLFCASDAKAYDTEVHNVWATHACVPTDPNPQEVVLVNVTENFNMWKNDMVEQMHEDIISLWDQSLKPCVKLTPLCVSLKCTDLKNDTNTNSSSGRMIMEKGEIKNCSFNISTSIRDKVQKEYAFFYKLDIVPIDNTSYRLISCNTSVITQACPKVSFEPIPIHYCAPAGFAILKCNNKTFNGTGPCTNVSTVQCTHGIRPVVSTQLLLNGSLAEEDVVIRSANFTDNAKTIIVQLNTSVEINCTRPNNNTRKSIRIQRGPGRAFVTIGKIGNMRQAHCNISRAKWNATLKQIASKLREQFGNNKTIIFKQSSGGDPEIVTHSFNCGGEFFYCNSTQLFNSTWFNSTWSTEGSNNTEGSDTITLPCRIKQFINMWQEVGKAMYAPPISGQIRCSSNITGLLLTRDGGNNNNGSEIFRPGGGDMRDNWRSELYKYKVVKIEPLGVAPTKKSLEQIWNNMTWMEWDREINNYTSLIHSLIEESQNQQEKNEQELLELDKWASLWNWFNITNWLWYIKLFIMIVGGLVGLRIVFAVLSIVNRVRQGYSPLSFQTHLPIPRGPDRPEGIEEEGGERDRDRSIRLVNGSLALIWDDLRSLCLFSYHRLRDLLLIVTRIVELLGRRGWEALKYWWNLLQYWSQELKNSAVNLLNATAIAVAEGTDRVIEVLQAAYRAIRHIPRRIRQGLERILL

SEQ ID NO: 18 - protein, 859 aa, Artificial Sequence
  BG505 gp160 (aa662-859 are transmembrane region and intracellular region)
MRVMGIQRNCQHLFRWGTMILGMIIICSAAENLWVTVYYGVPVWKDAETTLFCASDAKAYETEKHNVWATHACVPTDPNPQEIHLENVTEEFNMWKNNMVEQMHTDIISLWDQSLKPCVKLTPLCVTLQCTNVTNNITDDMRGELKNCSFNMTTELRDKKQKVYSLFYRLDVVQINENQGNRSNNSNKEYRLINCNTSAITQACPKVSFEPIPIHYCAPAGFAILKCKDKKFNGTGPCPSVSTVQCTHGIKPVVSTQLLLNGSLAEEEVMIRSENITNNAKNILVQFNTPVQINCTRPNNNTRKSIRIGPGQAFYATGDIIGDIRQAHCTVSKATWNETLGKVVKQLRKHFGNNTIIRFANSSGGDLEVTTHSFNCGGEFFYCNTSGLFNSTWISNTSVQGSNSTGSNDSITLPCRIKQIINMWQRIGQAMYAPPIQGVIRCVSNITGLILTRDGGSTNSTTETFRPGGGDMRDNWRSELYKYKVVKIEPLGVAPTRAKRRVVGREKRAVGIGAVFLGFLGAAGSTMGAASMTLTVQARNLLSGIVQQQSNLLRAIEAQQHLLKLTVWGIKQLQARVLAVERYLRDQQLLGIWGCSGKLICTTNVPWNSSWSNRNLSEIWDNMTWLQWDKEISNYTQIIYGLLEESQNQQEKNEQDLLALDKWASLWNWFDISNWLWYIKIFIMIVGGLIGLRIVFAVLSVIHRVRQGYSPLSFQTHTPNPRGLDRPERIEEEDGEQDRGRSTRLVSGFLALAWDDLRSLCLFCYHRLRDFILIAARIVELLGHSSLKGLRLGWEGLKYLWNLLAYWGRELKISAINLFDTIAIAVAEWTDRVIEIGQRLCRAFLHIPRRIRQGLERAL

SEQ ID NO: 19 - protein, 854 aa, Artificial Sequence
  NL4-3 gp160 (aa663-854 are transmembrane region and intracellular region)
MRVKEKYQHLWRWGWKWGTMLLGILMICSATEKLWVTVYYGVPVWKEATTTLFCASDAKAYDTEVHNVWATHACVPTDPNPQEVVLVNVTENFNMWKNDMVEQMHEDIISLWDQSLKPCVKLTPLCVSLKCTDLKNDTNTNSSSGRMIMEKGEIKNCSFNISTSIRDKVQKEYAFFYKLDIVPIDNTSYRLISCNTSVITQACPKVSFEPIPIHYCAPAGFAILKCNNKTFNGTGPCTNVSTVQCTHGIRPVVSTQLLLNGSLAEEDVVIRSANFTDNAKTIIVQLNTSVEINCTRPNNNTRKSIRIQRGPGRAFVTIGKIGNMRQAHCNISRAKWNATLKQIASKLREQFGNNKTIIFKQSSGGDPEIVTHSFNCGGEFFYCNSTQLFNSTWFNSTWSTEGSNNTEGSDTITLPCRIKQFINMWQEVGKAMYAPPISGQIRCSSNITGLLLTRDGGNNNNGSEIFRPGGGDMRDNWRSELYKYKVVKIEPLGVAPTKAKRRVVQREKRAVGIGALFLGFLGAAGSTMGAASMTLTVQARQLLSDIVQQQNNLLRAIEAQQHLLQLTVWGIKQLQARILAVERYLKDQQLLGIWGCSGKLICTTAVPWNASWSNKSLEQIWNNMTWMEWDREINNYTSLIHSLIEESQNQQEKNEQELLELDKWASLWNWFNITNWLWYIKLFIMIVGGLVGLRIVFAVLSIVNRVRQGYSPLSFQTHLPIPRGPDRPEGIEEEGGERDRDRSIRLVNGSLALIWDDLRSLCLFSYHRLRDLLLIVTRIVELLGRRGWEALKYWWNLLQYWSQELKNSAVNLLNATAIAVAEGTDRVIEVLQAAYRAIRHIPRRIRQGLERILL

SEQ ID NO: 20 - protein, 855 aa, Artificial Sequence
  25710 gp160 (aa657-855 are transmembrane region and intracellular region)
MRVRGTLRNYQQWWIWGVLGFWMLMICNVGGNLWVTVYYGVPVWKEATTTLFCASDAKAYDKEVHNVWATHACVPTDPNPQEMVLGNVTENFNMWKNEMVNQMHEDVISLWDQSLKPCVKLTPLCVTLECSNVTYNESMKEVKNCSFNLTTELRDKKQKVHALFYRLDIVPLNDTEKKNSSRPYRLINCNTSAITQACPKVTFDPIPIHYCTPAGYAILKCNDKKFNGTGPCHKVSTVQCTHGIKPVVSTQLLLNGSLAEGEIIIRSENLTNNAKTIIVHLNQSVEIVCARPSNNTRTSIRIGPGQTFYATGAITGDIRQAHCNISKDKWNETLQRVGEKLAEHFPNKTIKFNSSSGGDLEITTHSFNCRGEFFYCNTSGLFNGTFNGTYVSPNSTDSNSSSIITIPCRIKQIINMWQEVGRAMYAPPIAGNITCKSNITGLLLVRDGGTGSESNKTEIFRPGGGDMRDNWRSELYKYKVVEIKPLGVAPTKAKRRVVEREKRAVGIGAVFLGFLGAAGSTMGAASITLTVQARQLLSGIVQQQSNLLRAIEAQQHLLQLTVWGIKQLQTRVLAIERYLKDQQLLGIWGCSGKLICTTAVPWNYSWSNRSQDDIWDNMTWMQWDKEISNYTNTIYKLLEDSQIQQEKNEKDLLALDSWENLWNWFNITNWLWYIKIFIIIVGGLIGLRIIFAVLPIVNRVRQGYSPLSFQTHTPTPGGPDRLGRIEEEGGEQDNVRSIRLVNGFLALAWDDLRNLCLFSYHRLRDFILVAARVVELLGRNSLRGLQKGWEALKYLGSLVQYWGLELKRSAISLLDTIAIAVAEGTDRIIQLGQGICRAICNIPRRIRQGLEAALQ

SEQ ID NO: 21 - protein, 858 aa, Artificial Sequence
  X1632 gp160 (aa660-858 are transmembrane region and intracellular region)
MKVKGTQRDWHSLWNWGILILGLVIICSASNNLWVTVYYGVPVWEDADTTLFCASDAKAYSTESHNVWATHACVPTDPNPQEIYLENVTEDFNMWENNMVEQMQEDIISLWDESLKPCVKLTPLCVTLTCTNVTNVTDSVGTNSRLKGYKEELKNCSFNTTTEIRDKKKQEYALFYKLDIVPINDNSNNSNGYRLINCNVSTIKQACPKVSFDPIPIHYCAPAGFAILKCRDKEFNGTGTCRNVSTVQCTHGIKPVVSTQLLLNGSLAEGDIVIRSENITDNAKTIIVHLNKTVSITCTRPNNNTRKSIRIGPGQALYATGAIIGDTRQAHCNINGSEWYEMIQNVKNKLNETFKKNITFNPSSGGDLEITTHSFNCRGEFFYCNTSELFNSSHLFNGSTLSTNGTITLPCRIKQIVRMWQRVGQAMYAPPIAGNITCRSNITGLLLTRDGGTNKDTNEAETFRPGGGDMRDNWRSELYKYKVVKIKPLGVAPTRARRRVVEREKRAIGLGTVLLGFLGTAGSTMGAASITLTVQVRQLLSGIVQQQSNLLRAIEAQQHLLQLTVWGIKQLQARVLAVERYLKDQQILGIWGCSGKLICTTNVPWNSSWSNKSYSDIWDNLTWIQWEREISNYTQQIYTLLEESQNQQEKNEQELLALDKWASLWNWFDITNWLWYIKIFIMIVGGLIGLRIVFAVLSIINRVRKGYSPLSFQTLTRHQREPDRPGGIEEEDGEQDRDKSVRFVSGFLSPVWDDLRSLCLFSYRRLRDFILVAARTVELLGRSSLKGLRLGWEGLKYLWNLLLYWGRELKSSAINLLDTTAIAVANWTDRVIEVGQRIVRAFLHIPVRIRQGLERALL

SEQ ID NO: 22 - protein, 862 aa, Artificial Sequence
  CH119 gp160 (aa663-862 are transmembrane region and intracellular region)
MRVTGIRKNYRHLWRWGTMLLGMLMICSAVGNLWVTVYYGVPVWKEATTTLFCASDAKAYDTEVHNVWATHACVPTDPSPQELVLENVTENFNMWKNEMVNQMHEDVISLWDQSLKPCVKLTPLCVTLECSKVSNNETDKYNGTEEMKNCSFNATTVVRDRQQKVYALFYRLDIVPLTEKNSSENSSKYYRLINCNTSAITQACPKVSFEPIPIHYCTPAGYAILKCNDKTFNGTGPCHNVSTVQCTHGIKPVVSTQLLLNGSLAEGEIIIRSENLTNNVKTILVHLNQSVEIVCTRPNNNTRKSIRIGPGQTFYATGDIIGDIRQAHCNISKWHETLKRVSEKLAEHFPNKTINFTSSSGGDLEITTHSFTCRGEFFYCNTSGLFNSTYMPNGTYLHGDTNSNSSITIPCRIKQIINMWQEVGRAMYAPPIEGNITCKSNITGLLLVRDGGTESNNTETNNTEIFRPGGGDMRDNWRSELYKYKVVEIKPLGVAPTAAKRRVVEREKRAVGIGAVFLGFLGVAGSTMGAASMTLTVQARQLLSGIVQQQSNLLRAIEAQQHLLQLTVWGIKQLQTRVLAIERYLKDQQLLGIWGCSGKLICTTAVPWNSSWSNKSQKEIWDNMTWMQWDKEISNYTNTIYKLLEDSQNQQESNEKDLLALDSWNNLWNWFNITQWLWYIKIFIIIVGGLIGLRIIFAVLSIVNRVRQGYSPLSFQTLTPTSGGRPDRLERIEEEGGEQDRDRSIRLVNGFLALAWDDLRNLCLFSYHRLRDFILVAARVVELLGRTSLRGLQRGWEALKYLGSLVQYWGQELKKSAISLVDTIAIVVAEGTDRIIDIVQAFCRAIYNIPRRIRQGFEAALQ

SEQ ID NO: 23 - protein, 850 aa, Artificial Sequence
  CNE8 gp160 (aa652-850 are transmembrane region and intracellular region)
MRVKETQMNWPNLWKWGTLILGLVIICSASDNLWVTVYYGVPVWRDADTTLFCASDAKAYDTEVHNVWATHACVPTDPNPQEIHLENVTENFNMWKNKMAEQMQEDVISLWDESLKPCVQLTPLCVTLNCTNANLNATVNASTTIGNITDEVRNCSFNTTTELRDKKQNVYALFYKLDIVPINNNSEYRLINCNTSVIKQACPKVSFDPIPIHYCAPAGYAILRCNDKNFNGTGPCKNVSSVQCTHGIKPVVSTQLLLNGSLAEDEIIIRSENLTDNVKTIIVHLNKSVEINCTRPSNNTRTSVRIGPGQVFYRTGDIIGDIRKAYCEINRTKWHETLKQVATKLREHFNKTIIFQPPSGGDIEITMHHFNCRGEFFYCNTTKLFNSTWGENTTMEGHNDTIVLPCRIKQIVNMWQGVGQAMYAPPIRGSINCVSNITGILLTRDGGTNMSNETFRPGGGNIKDNWRSELYKYKVVEIEPLGIAPTKAKRRVVEREKRAVGIGAMIFGFLGAAGSTMGAASITLTVQARQLLSGIVQQQSNLLRAPEAQQHLLQLTVWGIKQLQARVLAVERYLKDQKFLGLWGCSGKIICTTAVPWNSTWSNRSYEEIWDNMTWIEWEREISNYTSQIYEILTESQNQQDRNEKDLLELDKWASLWNWFDITRWLWYIKIFIMIVGGLIGLRIIFAVLSIVNRVRQGYSPLSFQTPTHHQREPDRPERIEEGGGEQDRDRSVRLVSGFLALAWDDLRSLCLFSYHRLRDLILIAVRTVELLGHGGLKGLRRGWEGLKYLGNLLLYWGQELKISAISLLDATAIAVAGWTDRIIEVAQRAWRAILHIPRRIRQGLERSLL

SEQ ID NO: 24 - protein, 852 aa, Artificial Sequence
  p246F3 gp160 (aa654-852 are transmembrane region and intracellular region)
MRARGMLRTWQHWWIWGILGFWMLMICNMQDLWVTVYYGVPVWKDAKTTLFCASDAKAYEKEVHNVWATHACVPTDPNPQEIVMANVTEEFNMWKNNMVEQMHTDIISLWDQSLKPCVKLTPLCVTLDCKDYNYSITNNSTGMEGEIKNCSYNITTELRDKRQKVYSLFYRLDVVQINDSNDRNNSQYRLINCNTTTMTQACPKVTFDPIPIHYCAPAGFAILKCNNKTFNGKGPCNNVSSVQCTHGIKPVVSTQLLLNGSLAEKEIVIRSENLTDNVKTIIVHLNESVEINCTRPNNNTRKSVRIGPGQTFYATGDIIGNIRQAHCTVNKTEWNTALTRVSKKLKEYFPNKTIAFQPSSGGDLEITTFSFNCRGEFFYCNTSDLFNGTFNETSGQFNSTFNSTLQCRIKQIINMWQEVGQAMYAPPIAGSITCISNITGLILTRDGGNTNSTKETFRPGGGNMRDNWRSELYKYKVVKIEPLGVAPTKARRRVVEREKRAVGIGAVFIGFLGAAGSTMGAASITLTVQARQLLSGIVQQQSNLLRAIEAQQHLLKLTVWGIKQLQARVLAVERYLKDQQLLGIWGCSGKLICTTNVPWNSSWSNKSQDEIWDNMTWLQWDKEISNYTQIIYNLIEESQTQQELNERDLLALDKWANLWNWFDITKWLWYIKIFIMIVGGLIGLRIIFAVLSIVNRVRQGYSPLSFQTLTPNPRGPDRPGGIEEEGGEQGRNSYTRLVSGFLPLAWDDLRSLCLFSYHLLRDFILIAARAAELLGRSSLRGLQRGWETLKYLGSLVQYWGLELKKSAISLLDTIAIQVAEGTDRIIELIQGIYRAIRNIPRRIRQGAETALV

SEQ ID NO: 25 - protein, 853 aa, Artificial Sequence
  Bal.26 gp160 (aa662-853 are transmembrane region and intracellular region)
MRVTEIRKSYQHWWRWGIMLLGMLMICNAEEKLWVTVYYGVPVWKEATTTLFCASDAKAYDTEVHNVWATHACVPTDPNPQEVKMENVTENFNMWKNNVVEQMHEDIISLWDQSLKPCVKLTPLCVTLNCTDLKNATNGNNTNTTSSSGGMMGGGEMKNCSFNITTNIRGKVQKEYALFYELDIVPIDNKIDSYRLISCNTSVITQACPKVSFEPIPIHYCAPAGFAILKCKDKKFNGKGPCSNVSTVQCTHGIRPVVSTQLLLNGSLAEEEVVIRSENFTNNAKIIVVQLNESVEINCTRPNNNTRKSIHIGPGRAFYTTGEIIGDIRQAHCNLSRAKWNDTLNKIVIKLREQFGNKTIVFKHSSGGDPEIVTHSFNCGGEFFYCNSTQLFNSTWNVTEESNNTVENNTITLPCRIKQIINMWQEVGRAMYAPPIRGQIRCSSNITGLLLTRDGGPEDDKTEVFRPGGGDMRDNWRSELYKYKVVKIEPLGVAPTKAKRRVVQREKRAVGIGAVLLGFLGAAGSTMGAASMTLTVQARLLLSGIVQQQNNLLRAIEAQQHLLQLTVWGIKQLQARVLAVERYLRDQQLLGIWGCSGKLICTTAVPWNASWSNKSLNKIWDNMTWMEWDREINNYTSIIYSLIEESQNQQEKNEQELLELDKWASLWNWFDITKWLWYIKIFIMIVGGLIGLRIVFSVLSIVNRVRQGYSPLSFQTHLPASRGPDRPGGIEEEGGERDRDRSGPLVNGFLTLIWVDLRSLFLFSYHRLRDLLLIVTRIVELLGRRGWEVLKYWWNLLQYWSQELKNSAVSLLNTIAIAVAEGTDRVIEVVQRAVRAILHIPRRIRQGLERALL

SEQ ID NO: 26 - protein, 7 aa, Artificial Sequence
  BG505- deleted sequence from gp41
WNSSWSN

SEQ ID NO: 27 - protein, 11 aa, Artificial Sequence
  BG505- deleted sequence from gp120
AKRRVVGREKR

SEQ ID NO: 28 - protein, 5 aa, Artificial Sequence
  Linker-1
GGGGS

SEQ ID NO: 29 - protein, 10 aa, Artificial Sequence
  Linker-2
GGGGSGGGGS

SEQ ID NO: 30 - protein, 681 aa, Artificial Sequence
  BG-B1(1/1)
MDAMKRGLCCVLLLCGAVFVSPSQEIHARFRRGARAVGIGAVFLGFLGAAGSTMGAASMTLTVQARNLLSGIVQQQSNLLRAPEAQQHLLKLTVWGIKQLQARVLAVERYLRDQQLLGIWGCSGKLICTTNVPGGGGSAENLWVTVYYGVPVWKDAETTLFCASDAKAYETEKHNVWATHACVPTDPNPQEIHLENVTEEFNMWKNNMVEQMHTDIISLWDQSLKPCVKLTPLCVTLQCTNVTNNITDDMRGELKNCSFNMTTELRDKKQKVYSLFYRLDVVQINENQGNRSNNSNKEYRLINCNTSAITQACPKVSFEPIPIHYCAPAGFAILKCKDKKFNGTGPCPSVSTVQCTHGIKPVVSTQLLLNGSLAEEEVMIRSENITNNAKNILVQFNTPVQINCTRPNNNTRKSIRIGPGQAFYATGDIIGDIRQAHCNVSKATWNETLGKVVKQLRKHFGNNTIIRFANSSGGDLEVTTHSFNCGGEFFYCNTSGLFNSTWISNTSVQGSNSTGSNDSITLPCRIKQIINMWQRIGQAMYAPPIQGVIRCVSNITGLILTRDGGSTNSTTETFRPGGGDMRDNWRSELYKYKVVKIEPLGVAPTRAKRRVVGGGGGSWNSSWSNRNLSEIWDNMTWLQWDKEISNYTQIIYGLLEESQNQQEKNEQDLLALDHHHHHHHH

SEQ ID NO: 31 - protein, 686 aa, Artificial Sequence
  BG-B1(1/2)
MDAMKRGLCCVLLLCGAVFVSPSQEIHARFRRGARAVGIGAVFLGFLGAAGSTMGAASMTLTVQARNLLSGIVQQQSNLLRAPEAQQHLLKLTVWGIKQLQARVLAVERYLRDQQLLGIWGCSGKLICTTNVPGGGGSAENLWVTVYYGVPVWKDAETTLFCASDAKAYETEKHNVWATHACVPTDPNPQEIHLENVTEEFNMWKNNMVEQMHTDIISLWDQSLKPCVKLTPLCVTLQCTNVTNNITDDMRGELKNCSFNMTTELRDKKQKVYSLFYRLDVVQINENQGNRSNNSNKEYRLINCNTSAITQACPKVSFEPIPIHYCAPAGFAILKCKDKKFNGTGPCPSVSTVQCTHGIKPVVSTQLLLNGSLAEEEVMIRSENITNNAKNILVQFNTPVQINCTRPNNNTRKSIRIGPGQAFYATGDIIGDIRQAHCNVSKATWNETLGKVVKQLRKHFGNNTIIRFANSSGGDLEVTTHSFNCGGEFFYCNTSGLFNSTWISNTSVQGSNSTGSNDSITLPCRIKQIINMWQRIGQAMYAPPIQGVIRCVSNITGLILTRDGGSTNSTTETFRPGGGDMRDNWRSELYKYKVVKIEPLGVAPTRAKRRVVGGGGGSGGGGSWNSSWSNRNLSEIWDNMTWLQWDKEISNYTQIIYGLLEESQNQQEKNEQDLLALDHHHHHHHH

SEQ ID NO: 32 - protein, 691 aa, Artificial Sequence
  BG-B1(2/2)
MDAMKRGLCCVLLLCGAVFVSPSQEIHARFRRGARAVGIGAVFLGFLGAAGSTMGAASMTLTVQARNLLSGIVQQQSNLLRAPEAQQHLLKLTVWGIKQLQARVLAVERYLRDQQLLGIWGCSGKLICTTNVPGGGGSGGGGSAENLWVTVYYGVPVWKDAETTLFCASDAKAYETEKHNVWATHACVPTDPNPQEIHLENVTEEFNMWKNNMVEQMHTDIISLWDQSLKPCVKLTPLCVTLQCTNVTNNITDDMRGELKNCSFNMTTELRDKKQKVYSLFYRLDVVQINENQGNRSNNSNKEYRLINCNTSAITQACPKVSFEPIPIHYCAPAGFAILKCKDKKFNGTGPCPSVSTVQCTHGIKPVVSTQLLLNGSLAEEEVMIRSENITNNAKNILVQFNTPVQINCTRPNNNTRKSIRIGPGQAFYATGDIIGDIRQAHCNVSKATWNETLGKVVKQLRKHFGNNTIIRFANSSGGDLEVTTHSFNCGGEFFYCNTSGLFNSTWISNTSVQGSNSTGSNDSITLPCRIKQIINMWQRIGQAMYAPPIQGVIRCVSNITGLILTRDGGSTNSTTETFRPGGGDMRDNWRSELYKYKVVKIEPLGVAPTRAKRRVVGGGGGSGGGGSWNSSWSNRNLSEIWDNMTWLQWDKEISNYTQIIYGLLEESQNQQEKNEQDLLALDHHHHHHHH

SEQ ID NO: 33 - protein, 686 aa, Artificial Sequence
  BG-B1(2/1)
MDAMKRGLCCVLLLCGAVFVSPSQEIHARFRRGARAVGIGAVFLGFLGAAGSTMGAASMTLTVQARNLLSGIVQQQSNLLRAPEAQQHLLKLTVWGIKQLQARVLAVERYLRDQQLLGIWGCSGKLICTTNVPGGGGSGGGGSAENLWVTVYYGVPVWKDAETTLFCASDAKAYETEKHNVWATHACVPTDPNPQEIHLENVTEEFNMWKNNMVEQMHTDIISLWDQSLKPCVKLTPLCVTLQCTNVTNNITDDMRGELKNCSFNMTTELRDKKQKVYSLFYRLDVVQINENQGNRSNNSNKEYRLINCNTSAITQACPKVSFEPIPIHYCAPAGFAILKCKDKKFNGTGPCPSVSTVQCTHGIKPVVSTQLLLNGSLAEEEVMIRSENITNNAKNILVQFNTPVQINCTRPNNNTRKSIRIGPGQAFYATGDIIGDIRQAHCNVSKATWNETLGKVVKQLRKHFGNNTIIRFANSSGGDLEVTTHSFNCGGEFFYCNTSGLFNSTWISNTSVQGSNSTGSNDSITLPCRIKQIINMWQRIGQAMYAPPIQGVIRCVSNITGLILTRDGGSTNSTTETFRPGGGDMRDNWRSELYKYKVVKIEPLGVAPTRAKRRVVGGGGGSWNSSWSNRNLSEIWDNMTWLQWDKEISNYTQIIYGLLEESQNQQEKNEQDLLALDHHHHHHHH

SEQ ID NO: 34 - protein, 696 aa, Artificial Sequence
  BG-B1(2/3)
MDAMKRGLCCVLLLCGAVFVSPSQEIHARFRRGARAVGIGAVFLGFLGAAGSTMGAASMTLTVQARNLLSGIVQQQSNLLRAPEAQQHLLKLTVWGIKQLQARVLAVERYLRDQQLLGIWGCSGKLICTTNVPGGGGSGGGGSAENLWVTVYYGVPVWKDAETTLFCASDAKAYETEKHNVWATHACVPTDPNPQEIHLENVTEEFNMWKNNMVEQMHTDIISLWDQSLKPCVKLTPLCVTLQCTNVTNNITDDMRGELKNCSFNMTTELRDKKQKVYSLFYRLDVVQINENQGNRSNNSNKEYRLINCNTSAITQACPKVSFEPIPIHYCAPAGFAILKCKDKKFNGTGPCPSVSTVQCTHGIKPVVSTQLLLNGSLAEEEVMIRSENITNNAKNILVQFNTPVQINCTRPNNNTRKSIRIGPGQAFYATGDIIGDIRQAHCNVSKATWNETLGKVVKQLRKHFGNNTIIRFANSSGGDLEVTTHSFNCGGEFFYCNTSGLFNSTWISNTSVQGSNSTGSNDSITLPCRIKQIINMWQRIGQAMYAPPIQGVIRCVSNITGLILTRDGGSTNSTTETFRPGGGDMRDNWRSELYKYKVVKIEPLGVAPTRAKRRVVGGGGGSGGGGSGGGGSWNSSWSNRNLSEIWDNMTWLQWDKEISNYTQIIYGLLEESQNQQEKNEQDLLALDHHHHHHHH

SEQ ID NO: 35 - protein, 678 aa, Artificial Sequence
  BG-B2(1-1)
MDAMKRGLCCVLLLCGAVFVSPSQEIHARFRRGARAVGIGAVFLGFLGAAGSTMGAASMTLTVQARNLLSGIVQQQSNLLRAPEAQQHLLKLTVWGIKQLQARVLAVERYLRDQQLLGIWGCSGKLICTTNVPGGGGSLWVTVYYGVPVWKDAETTLFCASDAKAYETEKHNVWATHACVPTDPNPQEIHLENVTEEFNMWKNNMVEQMHTDIISLWDQSLKPCVKLTPLCVTLQCTNVTNNITDDMRGELKNCSFNMTTELRDKKQKVYSLFYRLDVVQINENQGNRSNNSNKEYRLINCNTSAITQACPKVSFEPIPIHYCAPAGFAILKCKDKKFNGTGPCPSVSTVQCTHGIKPVVSTQLLLNGSLAEEEVMIRSENITNNAKNILVQFNTPVQINCTRPNNNTRKSIRIGPGQAFYATGDIIGDIRQAHCNVSKATWNETLGKVVKQLRKHFGNNTIIRFANSSGGDLEVTTHSFNCGGEFFYCNTSGLFNSTWISNTSVQGSNSTGSNDSITLPCRIKQIINMWQRIGQAMYAPPIQGVIRCVSNITGLILTRDGGSTNSTTETFRPGGGDMRDNWRSELYKYKVVKIEPLGVAPTRAKRRVVGGGGGSWNSSWSNRNLSEIWDNMTWLQWDKEISNYTQIIYGLLEESQNQQEKNEQDLLALDHHHHHHHH

SEQ ID NO: 36 - protein, 684 aa, Artificial Sequence
  BG-B2(1-2)
MDAMKRGLCCVLLLCGAVFVSPSQEIHARFRRGARAVGIGAVFLGFLGAAGSTMGAASMTLTVQARNLLSGIVQQQSNLLRAPEAQQHLLKLTVWGIKQLQARVLAVERYLRDQQLLGIWGCSGKLICTTNVPGGGGSLWVTVYYGVPVWKDAETTLFCASDAKAYETEKHNVWATHACVPTDPNPQEIHLENVTEEFNMWKNNMVEQMHTDIISLWDQSLKPCVKLTPLCVTLQCTNVTNNITDDMRGELKNCSFNMTTELRDKKQKVYSLFYRLDVVQINENQGNRSNNSNKEYRLINCNTSAITQACPKVSFEPIPIHYCAPAGFAILKCKDKKFNGTGPCPSVSTVQCTHGIKPVVSTQLLLNGSLAEEEVMIRSENITNNAKNILVQFNTPVQINCTRPNNNTRKSIRIGPGQAFYATGDIIGDIRQAHCNVSKATWNETLGKVVKQLRKHFGNNTIIRFANSSGGDLEVTTHSFNCGGEFFYCNTSGLFNSTWISNTSVQGSNSTGSNDSITLPCRIKQIINMWQRIGQAMYAPPIQGVIRCVSNITGLILTRDGGSTNSTTETFRPGGGDMRDNWRSELYKYKVVKIEPLGVAPTRAKRRVVGGGGGSGGGGGSWNSSWSNRNLSEIWDNMTWLQWDKEISNYTQIIYGLLEESQNQQEKNEQDLLALDHHHHHHHH

SEQ ID NO: 37 - protein, 688 aa, Artificial Sequence
  BG-B2(1-3)
MDAMKRGLCCVLLLCGAVFVSPSQEIHARFRRGARAVGIGAVFLGFLGAAGSTMGAASMTLTVQARNLLSGIVQQQSNLLRAPEAQQHLLKLTVWGIKQLQARVLAVERYLRDQQLLGIWGCSGKLICTTNVPGGGGSLWVTVYYGVPVWKDAETTLFCASDAKAYETEKHNVWATHACVPTDPNPQEIHLENVTEEFNMWKNNMVEQMHTDIISLWDQSLKPCVKLTPLCVTLQCTNVTNNITDDMRGELKNCSFNMTTELRDKKQKVYSLFYRLDVVQINENQGNRSNNSNKEYRLINCNTSAITQACPKVSFEPIPIHYCAPAGFAILKCKDKKFNGTGPCPSVSTVQCTHGIKPVVSTQLLLNGSLAEEEVMIRSENITNNAKNILVQFNTPVQINCTRPNNNTRKSIRIGPGQAFYATGDIIGDIRQAHCNVSKATWNETLGKVVKQLRKHFGNNTIIRFANSSGGDLEVTTHSFNCGGEFFYCNTSGLFNSTWISNTSVQGSNSTGSNDSITLPCRIKQIINMWQRIGQAMYAPPIQGVIRCVSNITGLILTRDGGSTNSTTETFRPGGGDMRDNWRSELYKYKVVKIEPLGVAPTRAKRRVVGGGGGSGGGGSGGGGSWNSSWSNRNLSEIWDNMTWLQWDKEISNYTQIIYGLLEESQNQQEKNEQDLLALDHHHHHHHH

SEQ ID NO: 38 - protein, 681 aa, Artificial Sequence
  BG-C1(1/1)
MDAMKRGLCCVLLLCGAVFVSPSQEIHARFRRGARAVGIGAVFLGFLGAAGSTMGAASMTLTVQARNLLSGIVQQQSNLLRAPEAQQHLLKLTVWGIKQLQARVLAVERYLRDQQLLGIWGCSGKLICTTNVPWNSSWSNGGGGSAENLWVTVYYGVPVWKDAETTLFCASDAKAYETEKHNVWATHACVPTDPNPQEIHLENVTEEFNMWKNNMVEQMHTDIISLWDQSLKPCVKLTPLCVTLQCTNVTNNITDDMRGELKNCSFNMTTELRDKKQKVYSLFYRLDVVQINENQGNRSNNSNKEYRLINCNTSAITQACPKVSFEPIPIHYCAPAGFAILKCKDKKFNGTGPCPSVSTVQCTHGIKPVVSTQLLLNGSLAEEEVMIRSENITNNAKNILVQFNTPVQINCTRPNNNTRKSIRIGPGQAFYATGDIIGDIRQAHCNVSKATWNETLGKVVKQLRKHFGNNTIIRFANSSGGDLEVTTHSFNCGGEFFYCNTSGLFNSTWISNTSVQGSNSTGSNDSITLPCRIKQIINMWQRIGQAMYAPPIQGVIRCVSNITGLILTRDGGSTNSTTETFRPGGGDMRDNWRSELYKYKVVKIEPLGVAPTRAKRRVVGGGGGSRNLSEIWDNMTWLQWDKEISNYTQIIYGLLEESQNQQEKNEQDLLALDHHHHHHHH

SEQ ID NO: 39 - protein, 686 aa, Artificial Sequence
  BG-C1(1/2)
MDAMKRGLCCVLLLCGAVFVSPSQEIHARFRRGARAVGIGAVFLGFLGAAGSTMGAASMTLTVQARNLLSGIVQQQSNLLRAPEAQQHLLKLTVWGIKQLQARVLAVERYLRDQQLLGIWGCSGKLICTTNVPWNSSWSNGGGGSAENLWVTVYYGVPVWKDAETTLFCASDAKAYETEKHNVWATHACVPTDPNPQEIHLENVTEEFNMWKNNMVEQMHTDIISLWDQSLKPCVKLTPLCVTLQCTNVTNNITDDMRGELKNCSFNMTTELRDKKQKVYSLFYRLDVVQINENQGNRSNNSNKEYRLINCNTSAITQACPKVSFEPIPIHYCAPAGFAILKCKDKKFNGTGPCPSVSTVQCTHGIKPVVSTQLLLNGSLAEEEVMIRSENITNNAKNILVQFNTPVQINCTRPNNNTRKSIRIGPGQAFYATGDIIGDIRQAHCNVSKATWNETLGKVVKQLRKHFGNNTIIRFANSSGGDLEVTTHSFNCGGEFFYCNTSGLFNSTWISNTSVQGSNSTGSNDSITLPCRIKQIINMWQRIGQAMYAPPIQGVIRCVSNITGLILTRDGGSTNSTTETFRPGGGDMRDNWRSELYKYKVVKIEPLGVAPTRAKRRVVGGGGGSGGGGSRNLSEIWDNMTWLQWDKEISNYTQIIYGLLEESQNQQEKNEQDLLALDHHHHHHHH

SEQ ID NO: 40 - protein, 691 aa, Artificial Sequence
  BG-C1(1/3)
MDAMKRGLCCVLLLCGAVFVSPSQEIHARFRRGARAVGIGAVFLGFLGAAGSTMGAASMTLTVQARNLLSGIVQQQSNLLRAPEAQQHLLKLTVWGIKQLQARVLAVERYLRDQQLLGIWGCSGKLICTTNVPWNSSWSNGGGGSAENLWVTVYYGVPVWKDAETTLFCASDAKAYETEKHNVWATHACVPTDPNPQEIHLENVTEEFNMWKNNMVEQMHTDIISLWDQSLKPCVKLTPLCVTLQCTNVTNNITDDMRGELKNCSFNMTTELRDKKQKVYSLFYRLDVVQINENQGNRSNNSNKEYRLINCNTSAITQACPKVSFEPIPIHYCAPAGFAILKCKDKKFNGTGPCPSVSTVQCTHGIKPVVSTQLLLNGSLAEEEVMIRSENITNNAKNILVQFNTPVQINCTRPNNNTRKSIRIGPGQAFYATGDIIGDIRQAHCNVSKATWNETLGKVVKQLRKHFGNNTIIRFANSSGGDLEVTTHSFNCGGEFFYCNTSGLFNSTWISNTSVQGSNSTGSNDSITLPCRIKQIINMWQRIGQAMYAPPIQGVIRCVSNITGLILTRDGGSTNSTTETFRPGGGDMRDNWRSELYKYKVVKIEPLGVAPTRAKRRVVGGGGGSGGGGSGGGGSRNLSEIWDNMTWLQWDKEISNYTQIIYGLLEESQNQQEKNEQDLLALDHHHHHHHH

SEQ ID NO: 41 - protein, 4 aa, Artificial Sequence
  gp160 protein-furin cleavage site
REKR